European Patent Specification EP 4 028 559 B1, published January 7, 2026. Title: METHODS FOR DIAGNOSIS AND IN VITRO RISK STRATIFICATION FOR HEAD AND NECK CANCER BASED ON EXOSOMAL MRNAS. Applicant: Shrestha, Devjani Ghosh. Application 201931019425. The sequence listing filed with the application follows.

SEQUENCE LISTING (8 sequences)

SEQ ID NO: 1 - DNA, 456 bp, Human papillomavirus type 16
atgtttcaggacccacaggagcgacccagaaagttaccacagttatgcacagagctgcaaacaactatacatgatataatattagaatgtgtgtactgcaagcaacagttactgcgacgtgaggtatatgactttgcttttcgggatttatgcatagtatatagagatgggaatccatatgctgtatgtgataaatgtttaaagttttattctaaaattagtgagtatagacattattgttatagtttgtatggaacaacattagaacagcaatacaacaaaccgttgtgtgatttgttaattaggtgtattaactgtcaaaagccactgtgtcctgaagaaaagcaaagacatctggacaaaaagcaaagattccataatataaggggtcggtggaccggtcgatgtatgtcttgttgcagatcatcaagaacacgtagagaaacccagctgtaa

SEQ ID NO: 2 - DNA, 296 bp, Human papillomavirus type 16
atgcatggagatacacctacattgcatgaatatatgttagatttgcaaccagagacaactgatctctactgttatgagcaattaaatgacagctcagaggaggaggatgaaatagatggtccagctggacaagcagaaccggacagagcccattacaatattgtaaccttttgttgcaagtgtgactctacgctcggttgtgcgtacaaagcacacacgtagacattcgtactttggaagacctgttaatgggcacactaggaattgtgtgccccatctgttctcagaaaccataa

SEQ ID NO: 3 - DNA, 21 bp, Artificial Sequence
  Forward primer of primer set 1 (E6 primer)
gcgacccagaaagttaccaca

SEQ ID NO: 4 - DNA, 22 bp, Artificial Sequence
  Reverse primer of primer set 1 (E6 primer)
aagtcatatacctcacgtcgca

SEQ ID NO: 5 - DNA, 21 bp, Artificial Sequence
  Forward primer of primer set 2 (E7 primer)
cagaaccggacagagcccatt

SEQ ID NO: 6 - DNA, 22 bp, Artificial Sequence
  Reverse primer of primer set 2 (E7 primer)
aacagatggggcacacaattcc

SEQ ID NO: 7 - DNA, 22 bp, Artificial Sequence
  GAPDH Forward Primer
tcaccatcttccaggagcgaga

SEQ ID NO: 8 - DNA, 24 bp, Artificial Sequence
  GAPDH Reverse Primer
gcaggaggcattgctgatgatctt